European Patent Application EP 4 566 597 A1, published June 11, 2025. Title: STATINS USEFUL IN THE TREATMENT OF SPLACHNIC VASCULAR DYSFUNCTIONS. Applicant: HOSPITAL CLÍNIC DE BARCELONA. Application EP. The sequence listing filed with the application follows.

SEQUENCE LISTING (18 sequences)

SEQ ID NO: 1 - DNA, 20 bp, synthetic construct
  source 1..20: mol_type = other DNA
tcggagtcaacggatttggt

SEQ ID NO: 2 - DNA, 20 bp, synthetic construct
  source 1..20: mol_type = other DNA
ttcccgttctcagccttgac

SEQ ID NO: 3 - DNA, 20 bp, synthetic construct
  source 1..20: mol_type = other DNA
gaaagctgtccctgatgccg

SEQ ID NO: 4 - DNA, 20 bp, synthetic construct
  source 1..20: mol_type = other DNA
atgtccttccagggatgtgc

SEQ ID NO: 5 - DNA, 20 bp, synthetic construct
  source 1..20: mol_type = other DNA
cgagtgaaggcgacaatcct

SEQ ID NO: 6 - DNA, 20 bp, synthetic construct
  source 1..20: mol_type = other DNA
acaggacccggggatcaaaa

SEQ ID NO: 7 - DNA, 20 bp, synthetic construct
  source 1..20: mol_type = other DNA
aggcttctggtgaaatcgca

SEQ ID NO: 8 - DNA, 24 bp, synthetic construct
  source 1..24: mol_type = other DNA
gcagttgctaaacttcacattgag

SEQ ID NO: 9 - DNA, 19 bp, synthetic construct
  source 1..19: mol_type = other DNA
catggtgaggcaggtccag

SEQ ID NO: 10 - DNA, 20 bp, synthetic construct
  source 1..20: mol_type = other DNA
ggccacttgggagtgaatga

SEQ ID NO: 11 - DNA, 24 bp, synthetic construct
  source 1..24: mol_type = other DNA
tggataatgtttgcagcttctcaa

SEQ ID NO: 12 - DNA, 20 bp, synthetic construct
  source 1..20: mol_type = other DNA
agatgtggtcccctcattcg

SEQ ID NO: 13 - DNA, 22 bp, synthetic construct
  source 1..22: mol_type = other DNA
acctctgagaacttcaggatgc

SEQ ID NO: 14 - DNA, 20 bp, synthetic construct
  source 1..20: mol_type = other DNA
gggtgagaaaaccacgttgc

SEQ ID NO: 15 - DNA, 20 bp, synthetic construct
  source 1..20: mol_type = other DNA
ggccaaggagattgactcgg

SEQ ID NO: 16 - DNA, 19 bp, synthetic construct
  source 1..19: mol_type = other DNA
gcctcgtcgaacacggttt

SEQ ID NO: 17 - DNA, 20 bp, synthetic construct
  source 1..20: mol_type = other DNA
cgagtggttcttctgcgcta

SEQ ID NO: 18 - DNA, 22 bp, synthetic construct
  source 1..22: mol_type = other DNA
ctgctggaaggtaaactctgga